European Patent Application EP 4 718 075 A2, published April 1, 2026. Title: Antibodies recognizing genetic variants. Applicant: Roche Diagnostics GmbH. Application EP. The sequence listing filed with the application follows.

SEQUENCE LISTING (30 sequences)

SEQ ID NO: 1 - protein, 76 aa, Homo sapiens
  REGION 1..76: note = NT-proBNP with R46H mutation
HPLGSPGSASDLETSGLQEQRNHLQGKLSELQVEQTSLEPLQESPHPTGVWKSREVATEGIRGHRKMVLYTLRAPR

SEQ ID NO: 2 - protein, 76 aa, Homo sapiens
  REGION 1..76: note = NT-proBNP with E43D mutation
HPLGSPGSASDLETSGLQEQRNHLQGKLSELQVEQTSLEPLQDSPRPTGVWKSREVATEGIRGHRKMVLYTLRAPR

SEQ ID NO: 3 - protein, 76 aa, Homo sapiens
  REGION 1..76: note = wild-type NT-proBNP
HPLGSPGSASDLETSGLQEQRNHLQGKLSELQVEQTSLEPLQESPRPTGVWKSREVATEGIRGHRKMVLYTLRAPR

SEQ ID NO: 4 - protein, 212 aa, synthetic construct
  REGION 1..212: note = light chain of antibody S-22.2.195
YELTQPTSVSVALEQTAEITCQGDLLDDAYVAWYQQKPGQAPMKLIYKDSERPSGILDRFSGSSSGKIATLIISGARTEDEADYYCLSVDSSEYSVFGSGTRLTVLSQPKSAPSVTLFPPSKEELDTNKATVVCLISDFYPGSVNVVWKADGSTINQNVKTTQASKQSNSKYAASSYLTLTGSEWKSKSSYTCEVTHEGSTVTKTVKPSECS

SEQ ID NO: 5 - protein, 450 aa, synthetic construct
  REGION 1..450: note = heavy chain of antibody S-22.2.195
QVRLQESGPSLVKPSQTLSLTCTVSGFSLIGEYVTWVRQAPGKAPEWLSTMASGGTIFYNPTLKARLSITKDSTKSQFSLSVSSVTSEDTAMYYCVRSSVSPGDDRDVWGRGLLVTVSSASTTPPKVYPLTSCCGDTSSSIVTLGCLVSSYMPEPVTVTWNSGALTSGVHTFPAILQSSGLYSLSSVVTVPASTSGAQTFICNVAHPASSTKVDKRVEPGCPDPCKHCRCPPPELPGGPSVFIFPPKPKDTLTISGTPEVTCVVVDVGQDDPEVQFSWFVDNVEVRTARTKPREEQFNSTFRVVSALPIQHQDWTGGKEFKCKVHNEGLPAPIVRTISRTKGQAREPQVYVLAPPQEELSKSTLSVTCLVTGFYPDYIAVEWQKNGQPESEDKYGTTTSQLDADGSYFLYSRLRVDKNSWQEGDTYACVVMHEALHNHYTQKSISKPPGK

SEQ ID NO: 6 - protein, 7 aa, synthetic construct
  REGION 1..7: note = fragment of NT-proBNP with R46H mutation
ESPHPTG

SEQ ID NO: 7 - protein, 10 aa, synthetic construct
  REGION 1..10: note = fragment of NT-proBNP with R46H mutation
QESPHPTGVW

SEQ ID NO: 8 - protein, 7 aa, synthetic construct
  REGION 1..7: note = fragment of NT-proBNP with E43D mutation
PLQDSPR

SEQ ID NO: 9 - protein, 10 aa, synthetic construct
  REGION 1..10: note = fragment of NT-proBNP with E43D mutation
EPLQDSPRPT

SEQ ID NO: 10 - DNA, 636 bp, synthetic construct
  misc_feature 1..636: note = nucleic acid sequence for light chain of antibody S-22.2.195
  source 1..636: mol_type = other DNA
tatgaactgacccagccgacttcagtgtcggtggccttggaacagacggccgaaatcacctgccagggagatttgttggatgatgcatatgtggcttggtaccagcagaagccgggccaggctccgatgaaactcatttataaagacagtgagcggccttcagggatccttgaccggttctctggctccagctcaggcaaaatagccaccctaatcatcagcggggcccggaccgaggacgaggccgactattactgtctgtcagttgacagcagcgaatattctgttttcggcagcgggaccaggttgaccgttttgagtcagcccaagtccgcaccctcggtcaccctgttcccgccttccaaggaggagctcgataccaacaaggccaccgtggtgtgtctcatcagcgacttctacccgggtagcgtgaacgtggtctggaaggcagatggcagcaccatcaatcagaacgtgaagaccacccaggcctccaaacagagcaacagcaagtacgcggccagcagctacctgaccctgacgggcagcgagtggaagtctaagagcagttacacctgcgaggtcacgcacgaggggagcaccgtgacgaagacagtgaagccctcagagtgttct

SEQ ID NO: 11 - DNA, 1350 bp, synthetic construct
  misc_feature 1..1350: note = nucleic acid sequence for heavy chain of antibody S-22.2.195
  source 1..1350: mol_type = other DNA
caggtgcggctgcaggagtcgggacccagcctggtgaagccctcacagaccctctccctcacctgcacggtctctggattctcattaatcggcgagtatgtaacctgggtccgccaggctccaggaaaggcgccggagtggctgagtacgatggccagtggtggaaccatattttataatccgaccctgaaggcccgactcagcatcaccaaggacagcaccaagagccaattctccctgtcagtgagcagcgtgacatctgaggacacggccatgtattactgtgtaagatcttccgtttcaccgggcgatgatagagatgtctggggccgaggactcctggttaccgtctcctcggcctccaccacacccccgaaagtctaccctctgacttcttgctgcggggacacgtccagctccatcgtgaccctgggctgcctggtctccagctatatgcccgagccggtgaccgtgacctggaactctggtgccctgaccagcggcgtgcacaccttcccggccatcctgcagtcctccgggctctactctctcagcagcgtggtgaccgtgccggccagcacctcaggagcccagaccttcatctgcaacgtagcccacccggccagcagcaccaaggtggacaagcgtgttgagcccggatgcccggacccatgcaaacattgccgatgcccaccccctgagctccccggaggaccgtctgtcttcatcttcccaccgaaacccaaggacacccttacaatctctggaacgcccgaggtcacgtgtgtggtggtggacgtgggccaggatgaccccgaggtgcagttctcctggttcgtggacaacgtggaggtgcgcacggccaggacaaagccgagagaggagcagttcaacagcaccttccgcgtggtcagcgccctgcccatccagcaccaagactggactggaggaaaggagttcaagtgcaaggtccacaacgaaggcctcccggcccccatcgtgaggaccatctccaggaccaaagggcaggcccgggagccgcaggtgtacgtcctggccccaccccaggaagagctcagcaaaagcacgctcagcgtcacctgcctggtcaccggcttctacccagactacatcgccgtggagtggcagaaaaatgggcagcctgagtcggaggacaagtacggcacgaccacatcccagctggacgccgacggctcctacttcctgtacagcaggctcagggtggacaagaacagctggcaagaaggagacacctacgcgtgtgtggtgatgcacgaggctctgcacaaccactacacacagaagtcgatctctaagcctccgggtaaa

SEQ ID NO: 12 - protein, 217 aa, synthetic construct
  REGION 1..217: note = light chain of antibody S-23.4.66
QAVLTQPSSVSRSPGQSVSITCSGSSSNVGYGNYVGWFQQVPGSAPKLLIYSATSRASGVPDRFSGSRAGNTATLTITSLQAEDEADYYCVSYDSSSKFGVFGSGTRLTVLGQPKSAPSVTLFPPSTEELSTNKATVVCLINDFYPGSVNVVWKADGSTINQNVKTTQASKQSNSKYAASSYLTLTGSEWKSKSSYTCEVTHEGSTVTKTVKPSECS

SEQ ID NO: 13 - protein, 455 aa, synthetic construct
  REGION 1..455: note = heavy chain of antibody S-23.4.66
QVRMQELGPSLVKPSQTLSLTCTVSGFSVTNSGVGWVRQAPGKALEWLGIINNDGVAGYNPALKTRLSITRDTSKNQVSLSLSSVTTEDTAVYYCGTRDLPSDVRYGNMYINYWGPGRMVTVSSASTTPPKVYPLTSCCGDTSSSIVTLGCLVSSYMPEPVTVTWNSGALTSGVHTFPAILQSSGLYSLSSVVTVPASTSGAQTFICNVAHPASSTKVDKRVEPGCPDPCKHCRCPPPELPGGPSVFIFPPKPKDTLTISGTPEVTCVVVDVGQDDPEVQFSWFVDNVEVRTARTKPREEQFNSTFRVVSALPIQHQDWTGGKEFKCKVHNEGLPAPIVRTISRTKGQAREPQVYVLAPPQEELSKSTLSVTCLVTGFYPDYIAVEWQKNGQPESEDKYGTTTSQLDADGSYFLYSRLRVDKNSWQEGDTYACVVMHEALHNHYTQKSISKPPGK

SEQ ID NO: 14 - DNA, 651 bp, synthetic construct
  misc_feature 1..651: note = nucleic acid sequence for light chain of antibody S-23.4.66
  source 1..651: mol_type = other DNA
caggctgtgctgactcagccgtcctccgtgtccaggtccccgggccagagtgtctccatcacctgctctggaagcagcagcaacgttggatatggtaattatgtgggctggttccaacaagtcccaggatcagcccccaaactcctcatctatagtgcgaccagtcgagcctcgggggtccccgaccgattctccggctccagggctggcaacacagcgaccctgaccatcacttcgctccaggctgaggacgaggccgattattattgtgtatcttatgacagtagtagcaaatttggtgttttcggcagcgggaccaggctgaccgtcctgggtcagcccaagtccgcaccctcggtcaccctgttcccgccttccacggaggagctcagtaccaacaaggccaccgtggtgtgtctcatcaacgacttctacccgggtagcgtgaacgtggtctggaaggcagatggcagcaccatcaatcagaacgtgaagaccacccaggcctccaaacagagcaacagcaagtacgcggccagcagctacctgaccctgacgggcagcgagtggaagtctaagagcagttacacctgcgaggtcacgcacgaggggagcaccgtgacgaagacagtgaagccctcagagtgttct

SEQ ID NO: 15 - DNA, 1365 bp, synthetic construct
  misc_feature 1..1365: note = nucleic acid sequence for heavy chain of antibody S-23.4.66
  source 1..1365: mol_type = other DNA
caggtgcggatgcaggagttgggacccagcctggtgaagccctcacagaccctctccctcacgtgcacggtctctggattctcagtaaccaacagtggtgtaggctgggtccgccaggctccaggaaaggccctggagtggcttggtattataaataatgatggagtcgcaggctataacccagcccttaagacccggctcagcatcaccagggacacctccaagaaccaagtctccctgtcattgagcagcgtgacaactgaggacacggccgtgtactactgtggaacacgagatttgcccagtgatgttcgttatgggaacatgtatatcaactactggggcccaggacgaatggtcaccgtctcctcagcctccaccacacccccgaaagtctaccctctgacttcttgctgcggggacacgtccagctccatcgtgaccctgggctgcctggtctccagctatatgcccgagccggtgaccgtgacctggaactctggtgccctgaccagcggcgtgcacaccttcccggccatcctgcagtcctccgggctctactctctcagcagcgtggtgaccgtgccggccagcacctcaggagcccagaccttcatctgcaacgtagcccacccggccagcagcaccaaggtggacaagcgtgttgagcccggatgcccggacccatgcaaacattgccgatgcccaccccctgagctccccggaggaccgtctgtcttcatcttcccaccgaaacccaaggacacccttacaatctctggaacgcccgaggtcacgtgtgtggtggtggacgtgggccaggatgaccccgaggtgcagttctcctggttcgtggacaacgtggaggtgcgcacggccaggacaaagccgagagaggagcagttcaacagcaccttccgcgtggtcagcgccctgcccatccagcaccaagactggactggaggaaaggagttcaagtgcaaggtccacaacgaaggcctcccggcccccatcgtgaggaccatctccaggaccaaagggcaggcccgggagccgcaggtgtacgtcctggccccaccccaggaagagctcagcaaaagcacgctcagcgtcacctgcctggtcaccggcttctacccagactacatcgccgtggagtggcagaaaaatgggcagcctgagtcggaggacaagtacggcacgaccacatcccagctggacgccgacggctcctacttcctgtacagcaggctcagggtggacaagaacagctggcaagaaggagacacctacgcgtgtgtggtgatgcacgaggctctgcacaaccactacacacagaagtcgatctctaagcctccgggtaaa

SEQ ID NO: 16 - protein, 6 aa, synthetic construct
  REGION 1..6: note = CDR1 , light chain, antibody S-22.2.195
LLDDAY

SEQ ID NO: 17 - protein, 10 aa, synthetic construct
  REGION 1..10: note = CDR3, light chain, antibody S-22.2.195
LSVDSSEYSV

SEQ ID NO: 18 - protein, 8 aa, synthetic construct
  REGION 1..8: note = CDR1, heavy chain, antibody S-22.2.195
GFSLIGEY

SEQ ID NO: 19 - protein, 7 aa, synthetic construct
  REGION 1..7: note = CDR2, heavy chain, antibody S-22.2.195
MASGGTI

SEQ ID NO: 20 - protein, 13 aa, synthetic construct
  REGION 1..13: note = CDR3, heavy chain, antibody S-22.2.195
VRSSVSPGDDRDV

SEQ ID NO: 21 - protein, 9 aa, synthetic construct
  REGION 1..9: note = CDR1, light chain, antibody S-23.4.66
SSNVGYGNY

SEQ ID NO: 22 - protein, 11 aa, synthetic construct
  REGION 1..11: note = CDR3, light chain, antibody S-23.4.66
VSYDSSSKFGV

SEQ ID NO: 23 - protein, 8 aa, synthetic construct
  REGION 1..8: note = CDR1, heavy chain, antibody S-23.4.66
GFSVTNSG

SEQ ID NO: 24 - protein, 7 aa, synthetic construct
  REGION 1..7: note = CDR2, heavy chain, antibody S-23.4.66
INNDGVA

SEQ ID NO: 25 - protein, 18 aa, synthetic construct
  REGION 1..18: note = CDR3, heavy chain, antibody S-23.4.66
GTRDLPSDVRYGNMYINY

SEQ ID NO: 26 - protein, 92 aa, synthetic construct
  REGION 1..92: note = NT-proBNP with R46H mutation with additional sequences such as His tag
MRGSHPLGSPGSASDLETSGLQEQRNHLQGKLSELQVEQTSLEPLQESPRPTGVWKSREVATEGIRGHRKMVLYTLRAPRGGGSHHHHHHHH

SEQ ID NO: 27 - protein, 88 aa, synthetic construct
  REGION 1..88: note = NT-proBNP with R46H mutation with additional sequences such as His tag
HPLGSPGSASDLETSGLQEQRNHLQGKLSELQVEQTSLEPLQESPHPTGVWKSREVATEGIRGHRKMVLYTLRAPRGGGSHHHHHHHH

SEQ ID NO: 28 - protein, 92 aa, synthetic construct
  REGION 1..92: note = NT-proBNP with E43D mutation with additional sequences such as His tag
MRGSHPLGSPGSASDLETSGLQEQRNHLQGKLSELQVEQTSLEPLQDSPRPTGVWKSREVATEGIRGHRKMVLYTLRAPRGGGSHHHHHHHH

SEQ ID NO: 29 - protein, 4 aa, synthetic construct
  REGION 1..4: note = N-terminal sequence in fusion proteins
MRGS

SEQ ID NO: 30 - protein, 4 aa, synthetic construct
  REGION 1..4: note = C-terminal sequence in fusion proteins
GGGS